European Patent Specification EP 3 490 574 B1, published May 22, 2024. Title: EXPRESSION OF PTEN-LONG WITH OCOLYTIC VIRUSES. Applicant: Ohio State Innovation Foundation. The sequence listing filed with the application follows.

SEQUENCE LISTING (1 sequence)

SEQ ID NO: 1 - DNA, 1731 bp, Artificial Sequence [sequence omitted]